European Patent Specification EP 3 939 602 B1, published May 29, 2024. Title: LACTOBACILLUS SALIVARUS STRAIN AND ITS USE IN THE PREVENTION AND TREATMENT OF UROGENITAL TRACT DYSBIOSIS. Applicant: PROBISEARCH, S.L.U. The sequence listing filed with the application follows.

SEQUENCE LISTING (3 sequences)

SEQ ID NO: 1 - DNA, 20 bp, Artificial Sequence
  Primer pbl16
agagtttgatcctggctcag

SEQ ID NO: 2 - DNA, 20 bp, Artificial Sequence
  Primer mbl16
ggctgctggcacgtagttag

SEQ ID NO: 3 - DNA, 500 bp, Lactobacillus salivarius
aacgtcatcgatgaacagttactctcactcgtgttcttctctaacaacagagttttacgatccgaagaccttcttcactcacgcggcgttgctccatcagacttgcgtccattgtggaagattccctactgctgcctcccgtaggagtttgggccgtgtctcagtcccaatgtggccgatcaacctctcagttcggctacgtatcatcaccttggtaggccgttaccccaccaactagttaatacgccgcgggtccatctaaaagcgatagcagaaccatctttcatctaaggatcatgcgatccttatagatatacgggattagcacctgtttccaagtgttatccccttcttttaggcaggttacccacgtgttactcacccgtccgccactcaacttcttacggtgaatgcaagcattcggtgtaagaaagtttcgttcgacttgcatgtattaggcacgccgccagcgttcgtcctgagccaggagcaaactctca